European Patent Application EP 4 159 229 A1, published April 5, 2023. Title: Anti-Adrenomedullin (ADM) Binder for use in therapy or prevention of symptoms of illness. Applicant: AdrenoMed AG. Application EP. The sequence listing filed with the application follows.

SEQUENCE LISTING (23 sequences)

SEQ ID NO: 1 - protein, 52 aa, Homo sapiens
YRQSMNNFQGLRSFGCRFGTCTVQKLAHQIYQFTDKDKDNVAPRSKISPQGY

SEQ ID NO: 2 - protein, 11 aa, Homo sapiens
APRSKISPQGY

SEQ ID NO: 3 - protein, 22 aa, Homo sapiens
CTVQKLAHQIYQFTDKDKDNVA

SEQ ID NO: 4 - protein, 21 aa, Homo sapiens
YRQSMNNFQGLRSFGCRFGTC

SEQ ID NO: 5 - protein, 8 aa, Mus musculus
GYTFSRYW

SEQ ID NO: 6 - protein, 8 aa, Mus musculus
ILPGSGST

SEQ ID NO: 7 - protein, 11 aa, Mus musculus
TEGYEYDGFDY

SEQ ID NO: 8 - protein, 11 aa, Mus musculus
QSIVYSNGNTY

SEQ ID NO: 9 - protein, 9 aa, Mus musculus
FQGSHIPYT

SEQ ID NO: 10 - protein, 225 aa, synthetic construct
  REGION 1..225: note = AM-VH-C
QVQLQQSGAELMKPGASVKISCKATGYTFSRYWIEWVKQRPGHGLEWIGEILPGSGSTNYNEKFKGKATITADTSSNTAYMQLSSLTSEDSAVYYCTEGYEYDGFDYWGQGTTLTVSSASTKGPSVFPLAPSSKSTSGGTAALGCLVKDYFPEPVTVSWNSGALTSGVHTFPAVLQSSGLYSLSSVVTVPSSSLGTQTYICNVNHKPSNTKVDKRVEPKHHHHHH

SEQ ID NO: 11 - protein, 225 aa, synthetic construct
  REGION 1..225: note = AM-VH1
QVQLVQSGAEVKKPGSSVKVSCKASGYTFSRYWISWVRQAPGQGLEWMGRILPGSGSTNYAQKFQGRVTITADESTSTAYMELSSLRSEDTAVYYCTEGYEYDGFDYWGQGTTVTVSSASTKGPSVFPLAPSSKSTSGGTAALGCLVKDYFPEPVTVSWNSGALTSGVHTFPAVLQSSGLYSLSSVVTVPSSSLGTQTYICNVNHKPSNTKVDKRVEPKHHHHHH

SEQ ID NO: 12 - protein, 225 aa, synthetic construct
  REGION 1..225: note = AM-VH2-E40
QVQLVQSGAEVKKPGSSVKVSCKASGYTFSRYWIEWVRQAPGQGLEWMGRILPGSGSTNYAQKFQGRVTITADESTSTAYMELSSLRSEDTAVYYCTEGYEYDGFDYWGQGTTVTVSSASTKGPSVFPLAPSSKSTSGGTAALGCLVKDYFPEPVTVSWNSGALTSGVHTFPAVLQSSGLYSLSSVVTVPSSSLGTQTYICNVNHKPSNTKVDKRVEPKHHHHHH

SEQ ID NO: 13 - protein, 225 aa, synthetic construct
  REGION 1..225: note = AM-VH3-T26-E55
QVQLVQSGAEVKKPGSSVKVSCKATGYTFSRYWISWVRQAPGQGLEWMGEILPGSGSTNYAQKFQGRVTITADESTSTAYMELSSLRSEDTAVYYCTEGYEYDGFDYWGQGTTVTVSSASTKGPSVFPLAPSSKSTSGGTAALGCLVKDYFPEPVTVSWNSGALTSGVHTFPAVLQSSGLYSLSSVVTVPSSSLGTQTYICNVNHKPSNTKVDKRVEPKHHHHHH

SEQ ID NO: 14 - protein, 225 aa, synthetic construct
  REGION 1..225: note = AM-VH4-T26-E40-E55
QVQLVQSGAEVKKPGSSVKVSCKATGYTFSRYWIEWVRQAPGQGLEWMGEILPGSGSTNYAQKFQGRVTITADESTSTAYMELSSLRSEDTAVYYCTEGYEYDGFDYWGQGTTVTVSSASTKGPSVFPLAPSSKSTSGGTAALGCLVKDYFPEPVTVSWNSGALTSGVHTFPAVLQSSGLYSLSSVVTVPSSSLGTQTYICNVNHKPSNTKVDKRVEPKHHHHHH

SEQ ID NO: 15 - protein, 219 aa, synthetic construct
  REGION 1..219: note = AM-VL-C
DVLLSQTPLSLPVSLGDQATISCRSSQSIVYSNGNTYLEWYLQKPGQSPKLLIYRVSNRFSGVPDRFSGSGSGTDFTLKISRVEAEDLGVYYCFQGSHIPYTFGGGTKLEIKRTVAAPSVFIFPPSDEQLKSGTASVVCLLNNFYPREAKVQWKVDNALQSGNSQESVTEQDSKDSTYSLSSTLTLSKADYEKHKVYACEVTHQGLSSPVTKSFNRGEC

SEQ ID NO: 16 - protein, 219 aa, synthetic construct
  REGION 1..219: note = AM-VL1
DVVMTQSPLSLPVTLGQPASISCRSSQSIVYSNGNTYLNWFQQRPGQSPRRLIYRVSNRDSGVPDRFSGSGSGTDFTLKISRVEAEDVGVYYCFQGSHIPYTFGQGTKLEIKRTVAAPSVFIFPPSDEQLKSGTASVVCLLNNFYPREAKVQWKVDNALQSGNSQESVTEQDSKDSTYSLSSTLTLSKADYEKHKVYACEVTHQGLSSPVTKSFNRGEC

SEQ ID NO: 17 - protein, 219 aa, synthetic construct
  REGION 1..219: note = AM-VL2-E40
DVVMTQSPLSLPVTLGQPASISCRSSQSIVYSNGNTYLEWFQQRPGQSPRRLIYRVSNRDSGVPDRFSGSGSGTDFTLKISRVEAEDVGVYYCFQGSHIPYTFGQGTKLEIKRTVAAPSVFIFPPSDEQLKSGTASVVCLLNNFYPREAKVQWKVDNALQSGNSQESVTEQDSKDSTYSLSSTLTLSKADYEKHKVYACEVTHQGLSSPVTKSFNRGEC

SEQ ID NO: 18 - protein, 19 aa, Mus musculus
YRQSMNQGSRSNGCRFGTC

SEQ ID NO: 19 - protein, 12 aa, Mus musculus
CTFQKLAHQIYQ

SEQ ID NO: 20 - protein, 11 aa, Mus musculus
APRNKISPQGY

SEQ ID NO: 21 - protein, 12 aa, Homo sapiens
CTVQKLAHQIYQ

SEQ ID NO: 22 - protein, 448 aa, synthetic construct
  REGION 1..448: note = Human antibody heavy chain with grafted mouse CDR
QVQLVQSGAEVKKPGSSVKVSCKASGYTFSRYWIEWVRQAPGQGLEWIGEILPGSGSTNYNQKFQGRVTITADTSTSTAYMELSSLRSEDTAVYYCTEGYEYDGFDYWGQGTTVTVSSASTKGPSVFPLAPSSKSTSGGTAALGCLVKDYFPEPVTVSWNSGALTSGVHTFPAVLQSSGLYSLSSVVTVPSSSLGTQTYICNVNHKPSNTKVDKKVEPKSCDKTHTCPPCPAPELLGGPSVFLFPPKPKDTLMISRTPEVTCVVVDVSHEDPEVKFNWYVDGVEVHNAKTKPREEQYNSTYRVVSVLTVLHQDWLNGKEYKCKVSNKALPAPIEKTISKAKGQPREPQVYTLPPSRDELTKNQVSLTCLVKGFYPSDIAVEWESNGQPENNYKTTPPVLDSDGSFFLYSKLTVDKSRWQQGNVFSCSVMHEALHNHYTQKSLSLSPGK

SEQ ID NO: 23 - protein, 219 aa, synthetic construct
  REGION 1..219: note = Human antibody light chain with grafted mouse CDRs
DVVLTQSPLSLPVTLGQPASISCRSSQSIVYSNGNTYLEWYLQRPGQSPRLLIYRVSNRFSGVPDRFSGSGSGTDFTLKISRVEAEDVGVYYCFQGSHIPYTFGGGTKLEIKRTVAAPSVFIFPPSDEQLKSGTASVVCLLNNFYPREAKVQWKVDNALQSGNSQESVTEQDSKDSTYSLSSTLTLSKADYEKHKVYACEVTHQGLSSPVTKSFNRGEC